European Patent Specification EP 3 489 253 B1, published March 1, 2023. Title: A novel peptide and use thereof. Applicant: ENSOL BIOSCIENCES INC. The sequence listing filed with the application follows.

SEQUENCE LISTING (4 sequences)

SEQ ID NO: 1 - protein, 5 aa, Artificial Sequence
  peptide
DGEFF

SEQ ID NO: 2 - protein, 4 aa, Artificial Sequence
  peptide
DGEF

SEQ ID NO: 3 - protein, 4 aa, Artificial Sequence
  peptide
DAEF

SEQ ID NO: 4 - protein, 8 aa, Artificial Sequence
  peptide
VKMDAEFR